European Patent Specification EP 4 001 428 B1, published November 22, 2023. Title: METHOD FOR REDUCING PRIMER DIMER FORMATION AND INCREASING AMPLIFICATION EFFICIENCY. Applicant: SEEGENE, INC. The sequence listing filed with the application follows.

SEQUENCE LISTING (62 sequences)

SEQ ID NO: 1 - DNA, 24 bp, Artificial Sequence
  Synthetic oligonucleotide: UP-R1
ggttctcaagcaacaatatcagct

SEQ ID NO: 2 - DNA, 11 bp, Artificial Sequence
  Synthetic oligonucleotide: UP-N-1
agctgatattg

SEQ ID NO: 3 - DNA, 13 bp, Artificial Sequence
  Synthetic oligonucleotide: UP-N-2
agctgatattgtt

SEQ ID NO: 4 - DNA, 15 bp, Artificial Sequence
  Synthetic oligonucleotide: UP-N-3
agctgatattgttgc

SEQ ID NO: 5 - DNA, 22 bp, Artificial Sequence
  Synthetic oligonucleotide: UP-P-1
ttggcttggcttggcttagctg

SEQ ID NO: 6 - DNA, 24 bp, Artificial Sequence
  Synthetic oligonucleotide: UP-P-2
ttggcttggcttggcttagctgat

SEQ ID NO: 7 - DNA, 26 bp, Artificial Sequence
  Synthetic oligonucleotide: UP-P-3
ttggcttggcttggcttagctgatat

SEQ ID NO: 8 - DNA, 21 bp, Artificial Sequence
  Synthetic oligonucleotide: UP-C-1
ttggcttggcttggcttagct

SEQ ID NO: 9 - DNA, 22 bp, Artificial Sequence
  Synthetic oligonucleotide: UP-C-2
ttggcttggcttggcttagctg

SEQ ID NO: 10 - DNA, 23 bp, Artificial Sequence
  Synthetic oligonucleotide: UP-C-3
ttggcttggcttggcttagctga

SEQ ID NO: 11 - DNA, 24 bp, Artificial Sequence
  Synthetic oligonucleotide: UP-C-4
ttggcttggcttggcttagctgat

SEQ ID NO: 12 - DNA, 21 bp, Artificial Sequence
  Synthetic oligonucleotide: NG-F4
gcggacagttgtttttcgact

SEQ ID NO: 13 - DNA, 11 bp, Artificial Sequence
  Synthetic oligonucleotide: NG-N-1
agtcgaaaaac

SEQ ID NO: 14 - DNA, 13 bp, Artificial Sequence
  Synthetic oligonucleotide: NG-N-2
agtcgaaaaacaa

SEQ ID NO: 15 - DNA, 15 bp, Artificial Sequence
  Synthetic oligonucleotide: NG-N-3
agtcgaaaaacaact

SEQ ID NO: 16 - DNA, 22 bp, Artificial Sequence
  Synthetic oligonucleotide: NG-P-1
ttggcttggcttggcttagtcg

SEQ ID NO: 17 - DNA, 24 bp, Artificial Sequence
  Synthetic oligonucleotide: NG-P-2
ttggcttggcttggcttagtcgaa

SEQ ID NO: 18 - DNA, 26 bp, Artificial Sequence
  Synthetic oligonucleotide: NG-P-3
ttggcttggcttggcttagtcgaaaa

SEQ ID NO: 19 - DNA, 21 bp, Artificial Sequence
  Synthetic oligonucleotide: NG-C-1
ttggcttggcttggcttagtc

SEQ ID NO: 20 - DNA, 22 bp, Artificial Sequence
  Synthetic oligonucleotide: NG-C-2
ttggcttggcttggcttagtcg

SEQ ID NO: 21 - DNA, 23 bp, Artificial Sequence
  Synthetic oligonucleotide: NG-C-3
ttggcttggcttggcttagtcga

SEQ ID NO: 22 - DNA, 24 bp, Artificial Sequence
  Synthetic oligonucleotide: NG-C-4
ttggcttggcttggcttagtcgaa

SEQ ID NO: 23 - DNA, 24 bp, Artificial Sequence
  Synthetic oligonucleotide: UP-F1
gcacaatttggatcattaaaaggt

SEQ ID NO: 24 - DNA, 20 bp, Artificial Sequence
  Synthetic oligonucleotide: NG-R2
gtcgtatccgcatccgtcaa

SEQ ID NO: 25 - DNA, 25 bp, Artificial Sequence
  Synthetic oligonucleotide: UP-P1
cccagctattgcacatggtgttgat

SEQ ID NO: 26 - DNA, 22 bp, Artificial Sequence
  Synthetic oligonucleotide: NG-P2
tgtacggctccgttgtggcggt

SEQ ID NO: 27 - DNA, 24 bp, Artificial Sequence
  Synthetic oligonucleotide: UP-IR-2
  misc_feature (23): n is deoxyinosine
ggttctcaagcaacaatatcagnt

SEQ ID NO: 28 - DNA, 24 bp, Artificial Sequence
  Synthetic oligonucleotide: UP-IR-3
  misc_feature (22): n is deoxyinosine
ggttctcaagcaacaatatcanct

SEQ ID NO: 29 - DNA, 24 bp, Artificial Sequence
  Synthetic oligonucleotide: UP-IR-4
  misc_feature (21): n is deoxyinosine
ggttctcaagcaacaatatcngct

SEQ ID NO: 30 - DNA, 24 bp, Artificial Sequence
  Synthetic oligonucleotide: UP-IR-5
  misc_feature (20): n is deoxyinosine
ggttctcaagcaacaatatnagct

SEQ ID NO: 31 - DNA, 24 bp, Artificial Sequence
  Synthetic oligonucleotide: UP-IR-6
  misc_feature (19): n is deoxyinosine
ggttctcaagcaacaatancagct

SEQ ID NO: 32 - DNA, 24 bp, Artificial Sequence
  Synthetic oligonucleotide: UP-IR-7
  misc_feature (18): n is deoxyinosine
ggttctcaagcaacaatntcagct

SEQ ID NO: 33 - DNA, 24 bp, Artificial Sequence
  Synthetic oligonucleotide: UP-IR-8
  misc_feature (17): n is deoxyinosine
ggttctcaagcaacaanatcagct

SEQ ID NO: 34 - DNA, 21 bp, Artificial Sequence
  Synthetic oligonucleotide: NG-IF-2
  misc_feature (20): n is deoxyinosine
gcggacagttgtttttcgant

SEQ ID NO: 35 - DNA, 21 bp, Artificial Sequence
  Synthetic oligonucleotide: NG-IF-3
  misc_feature (19): n is deoxyinosine
gcggacagttgtttttcgnct

SEQ ID NO: 36 - DNA, 21 bp, Artificial Sequence
  Synthetic oligonucleotide: NG-IF-4
  misc_feature (18): n is deoxyinosine
gcggacagttgtttttcnact

SEQ ID NO: 37 - DNA, 21 bp, Artificial Sequence
  Synthetic oligonucleotide: NG-IF-5
  misc_feature (17): n is deoxyinosine
gcggacagttgtttttngact

SEQ ID NO: 38 - DNA, 21 bp, Artificial Sequence
  Synthetic oligonucleotide: NG-IF-6
  misc_feature (16): n is deoxyinosine
gcggacagttgttttncgact

SEQ ID NO: 39 - DNA, 21 bp, Artificial Sequence
  Synthetic oligonucleotide: NG-IF-7
  misc_feature (15): n is deoxyinosine
gcggacagttgtttntcgact

SEQ ID NO: 40 - DNA, 21 bp, Artificial Sequence
  Synthetic oligonucleotide: NG-IF-8
  misc_feature (14): n is deoxyinosine
gcggacagttgttnttcgact

SEQ ID NO: 41 - DNA, 28 bp, Artificial Sequence
  Synthetic oligonucleotide: UU-F1
gcatatgatgaagcacacaacaaaatgg

SEQ ID NO: 42 - DNA, 22 bp, Artificial Sequence
  Synthetic oligonucleotide: UU-R1
gctttggctgatgattgcgtag

SEQ ID NO: 43 - DNA, 22 bp, Artificial Sequence
  Synthetic oligonucleotide: MG-F1
aaaacccacggaaatgatgaga

SEQ ID NO: 44 - DNA, 26 bp, Artificial Sequence
  Synthetic oligonucleotide: MG-R1
ctcgttaatttacctattccattttg

SEQ ID NO: 45 - DNA, 20 bp, Artificial Sequence
  Synthetic oligonucleotide: NG-F1
tacgcctgctactttcacgc

SEQ ID NO: 46 - DNA, 21 bp, Artificial Sequence
  Synthetic oligonucleotide: NG-R1
caatggatcggtatcactcgc

SEQ ID NO: 47 - DNA, 27 bp, Artificial Sequence
  Synthetic oligonucleotide: CT-F1
ttattcatccgaatggataaagcgtga

SEQ ID NO: 48 - DNA, 22 bp, Artificial Sequence
  Synthetic oligonucleotide: CT-R1
aacaatgaatcctgagcaaagg

SEQ ID NO: 49 - DNA, 28 bp, Artificial Sequence
  Synthetic oligonucleotide: UU-F2
  misc_feature (26): n is deoxyinosine
gcatatgatgaagcacacaacaaaangg

SEQ ID NO: 50 - DNA, 22 bp, Artificial Sequence
  Synthetic oligonucleotide: MG-F2
  misc_feature (18): n is deoxyinosine
aaaacccacggaaatgangaga

SEQ ID NO: 51 - DNA, 20 bp, Artificial Sequence
  Synthetic oligonucleotide: NG-F2
  misc_feature (17): n is deoxyinosine
tacgcctgctactttcncgc

SEQ ID NO: 52 - DNA, 27 bp, Artificial Sequence
  Synthetic oligonucleotide: CT-F2
  misc_feature (25): n is deoxyinosine
ttattcatccgaatggataaagcgnga

SEQ ID NO: 53 - DNA, 28 bp, Artificial Sequence
  Synthetic oligonucleotide: UU-F3
  misc_feature (13): n is deoxyinosine
  misc_feature (26): n is deoxyinosine
gcatatgatgaancacacaacaaaangg

SEQ ID NO: 54 - DNA, 22 bp, Artificial Sequence
  Synthetic oligonucleotide: MG-F3
  misc_feature (10): n is deoxyinosine
  misc_feature (18): n is deoxyinosine
aaaacccacngaaatgangaga

SEQ ID NO: 55 - DNA, 20 bp, Artificial Sequence
  Synthetic oligonucleotide: NG-F3
  misc_feature (10): n is deoxyinosine
  misc_feature (17): n is deoxyinosine
tacgcctgcnactttcncgc

SEQ ID NO: 56 - DNA, 27 bp, Artificial Sequence
  Synthetic oligonucleotide: CT-F3
  misc_feature (14): n is deoxyinosine
  misc_feature (25): n is deoxyinosine
ttattcatccgaanggataaagcgnga

SEQ ID NO: 57 - DNA, 27 bp, Artificial Sequence
  UU-P1
cacttcaccagatacataacccccgcc

SEQ ID NO: 58 - DNA, 28 bp, Artificial Sequence
  MG-P1
acacctcttgctgttcttgaaagaactc

SEQ ID NO: 59 - DNA, 22 bp, Artificial Sequence
  NG-P1
tgcccctcattggcgtgtttcg

SEQ ID NO: 60 - DNA, 29 bp, Artificial Sequence
  CT-P1
cattgtaaagatatggtctgcttcgaccg

SEQ ID NO: 61 - DNA, 17 bp, Artificial Sequence
  primer
  misc_feature 3..15: /note="n is any nucleotide"
agnnnnnnnnnnnnnct

SEQ ID NO: 62 - DNA, 26 bp, Artificial Sequence
  primer
aaaaaaaaaaaaaaaaaaaaggggaa